European Patent Application EP 4 119 665 A1, published January 18, 2023. Title: siRNA based on RNA sequence of SARS-CoV-2 and use thereof. Applicant: TOAGOSEI CO., LTD. The sequence listing filed with the application follows.

SEQUENCE LISTING (42 sequences)

SEQ ID NO: 1 - RNA, 19 nt, synthetic construct
  misc_feature 1..19: note = target sequence in siRNA
  source 1..19: mol_type = other RNA
gttttattgccactagtct

SEQ ID NO: 2 - RNA, 19 nt, synthetic construct
  misc_feature 1..19: note = target sequence in siRNA
  source 1..19: mol_type = other RNA
gtctctagtcagtgtgtta

SEQ ID NO: 3 - RNA, 19 nt, synthetic construct
  misc_feature 1..19: note = target sequence in siRNA
  source 1..19: mol_type = other RNA
cagtgtgttaatcttacaa

SEQ ID NO: 4 - protein, 16 aa, Severe acute respiratory syndrome coronavirus 2
MFVFLVLLPLVSSQCV

SEQ ID NO: 5 - RNA, 48 nt, Severe acute respiratory syndrome coronavirus 2
  source 1..48: mol_type = viral cRNA
atgtttgtttttcttgttttattgccactagtctctagtcagtgtgtt

SEQ ID NO: 6 - DNA, 21 bp, synthetic construct
  misc_feature 1..19: note = RNA
  source 1..21: mol_type = other DNA
  modified_base 2..5: mod_base = OTHER; note = uracil
  modified_base 7..8: mod_base = OTHER; note = uracil
  modified_base 14: mod_base = OTHER; note = uracil
  modified_base 17: mod_base = OTHER; note = uracil
  modified_base 19: mod_base = OTHER; note = uracil
  misc_feature 20..21: note = DNA
gttttattgccactagtcttt

SEQ ID NO: 7 - DNA, 21 bp, synthetic construct
  misc_feature 1..19: note = RNA
  source 1..21: mol_type = other DNA
  modified_base 5: mod_base = OTHER; note = uracil
  modified_base 8: mod_base = OTHER; note = uracil
  modified_base 14: mod_base = OTHER; note = uracil
  misc_feature 20..21: note = DNA
agactagtggcaataaaactt

SEQ ID NO: 8 - DNA, 21 bp, synthetic construct
  misc_feature 1..19: note = RNA
  source 1..21: mol_type = other DNA
  modified_base 2: mod_base = OTHER; note = uracil
  modified_base 4: mod_base = OTHER; note = uracil
  modified_base 6: mod_base = OTHER; note = uracil
  modified_base 9: mod_base = OTHER; note = uracil
  modified_base 13: mod_base = OTHER; note = uracil
  modified_base 15: mod_base = OTHER; note = uracil
  modified_base 17..18: mod_base = OTHER; note = uracil
  misc_feature 20..21: note = DNA
gtctctagtcagtgtgttatt

SEQ ID NO: 9 - DNA, 21 bp, synthetic construct
  misc_feature 1..19: note = RNA
  source 1..21: mol_type = other DNA
  modified_base 1: mod_base = OTHER; note = uracil
  modified_base 9: mod_base = OTHER; note = uracil
  modified_base 13: mod_base = OTHER; note = uracil
  misc_feature 20..21: note = DNA
taacacactgactagagactt

SEQ ID NO: 10 - DNA, 21 bp, synthetic construct
  misc_feature 1..19: note = RNA
  source 1..21: mol_type = other DNA
  modified_base 4: mod_base = OTHER; note = uracil
  modified_base 6: mod_base = OTHER; note = uracil
  modified_base 8..9: mod_base = OTHER; note = uracil
  modified_base 12: mod_base = OTHER; note = uracil
  modified_base 14..15: mod_base = OTHER; note = uracil
  misc_feature 20..21: note = DNA
cagtgtgttaatcttacaatt

SEQ ID NO: 11 - DNA, 21 bp, synthetic construct
  misc_feature 1..19: note = RNA
  source 1..21: mol_type = other DNA
  modified_base 1..2: mod_base = OTHER; note = uracil
  modified_base 4: mod_base = OTHER; note = uracil
  modified_base 9..10: mod_base = OTHER; note = uracil
  modified_base 18: mod_base = OTHER; note = uracil
  misc_feature 20..21: note = DNA
ttgtaagattaacacactgtt

SEQ ID NO: 12 - DNA, 21 bp, synthetic construct
  misc_feature 1..19: note = RNA
  source 1..21: mol_type = other DNA
  modified_base 2..5: mod_base = OTHER; note = uracil
  modified_base 7..8: mod_base = OTHER; note = uracil
  modified_base 14: mod_base = OTHER; note = uracil
  modified_base 17: mod_base = OTHER; note = uracil
  misc_feature 20..21: note = DNA
gttttcttaggaatcatcatt

SEQ ID NO: 13 - DNA, 21 bp, synthetic construct
  misc_feature 1..19: note = RNA
  source 1..21: mol_type = other DNA
  modified_base 1: mod_base = OTHER; note = uracil
  modified_base 4: mod_base = OTHER; note = uracil
  modified_base 7..8: mod_base = OTHER; note = uracil
  modified_base 11: mod_base = OTHER; note = uracil
  misc_feature 20..21: note = DNA
tgatgattcctaagaaaactt

SEQ ID NO: 14 - DNA, 21 bp, synthetic construct
  misc_feature 1..19: note = RNA
  source 1..21: mol_type = other DNA
  modified_base 3: mod_base = OTHER; note = uracil
  modified_base 7..9: mod_base = OTHER; note = uracil
  modified_base 19: mod_base = OTHER; note = uracil
  misc_feature 20..21: note = DNA
gctgcatttcaccaagaattt

SEQ ID NO: 15 - DNA, 21 bp, synthetic construct
  misc_feature 1..19: note = RNA
  source 1..21: mol_type = other DNA
  modified_base 2..3: mod_base = OTHER; note = uracil
  modified_base 5..6: mod_base = OTHER; note = uracil
  modified_base 9: mod_base = OTHER; note = uracil
  modified_base 14: mod_base = OTHER; note = uracil
  misc_feature 20..21: note = DNA
attcttggtgaaatgcagctt

SEQ ID NO: 16 - DNA, 21 bp, synthetic construct
  misc_feature 1..19: note = RNA
  source 1..21: mol_type = other DNA
  modified_base 7: mod_base = OTHER; note = uracil
  modified_base 9: mod_base = OTHER; note = uracil
  modified_base 12..14: mod_base = OTHER; note = uracil
  modified_base 19: mod_base = OTHER; note = uracil
  misc_feature 20..21: note = DNA
caagaatgtagtttacagttt

SEQ ID NO: 17 - DNA, 21 bp, synthetic construct
  misc_feature 1..19: note = RNA
  source 1..21: mol_type = other DNA
  modified_base 3: mod_base = OTHER; note = uracil
  modified_base 5: mod_base = OTHER; note = uracil
  modified_base 10: mod_base = OTHER; note = uracil
  modified_base 14..15: mod_base = OTHER; note = uracil
  modified_base 17..18: mod_base = OTHER; note = uracil
  misc_feature 20..21: note = DNA
actgtaaactacattcttgtt

SEQ ID NO: 18 - RNA, 45 nt, Severe acute respiratory syndrome coronavirus 2
  source 1..45: mol_type = viral cRNA
atgaaatttcttgttttcttaggaatcatcacaactgtagctgca

SEQ ID NO: 19 - DNA, 20 bp, synthetic construct
  misc_feature 1..20: note = PCR_primers_fwd_seq
  source 1..20: mol_type = other DNA
cttccctcagtcagcacctc

SEQ ID NO: 20 - DNA, 20 bp, synthetic construct
  misc_feature 1..20: note = PCR_primers_rev_seq
  source 1..20: mol_type = other DNA
aaccagtgtgtgccatttga

SEQ ID NO: 21 - DNA, 20 bp, synthetic construct
  misc_feature 1..20: note = PCR_primers_fwd_seq
  source 1..20: mol_type = other DNA
gctgcatttcaccaagaatg

SEQ ID NO: 22 - DNA, 20 bp, synthetic construct
  misc_feature 1..20: note = PCR_primers_rev_seq
  source 1..20: mol_type = other DNA
ctcatccacgcacaattcaa

SEQ ID NO: 23 - DNA, 23 bp, synthetic construct
  misc_feature 1..23: note = PCR_primers_fwd_seq
  source 1..23: mol_type = other DNA
cactttgcttcacactcaaaaga

SEQ ID NO: 24 - DNA, 22 bp, synthetic construct
  misc_feature 1..22: note = PCR_primers_rev_seq
  source 1..22: mol_type = other DNA
cattcttggtgaaatgcagcta

SEQ ID NO: 25 - DNA, 26 bp, synthetic construct
  misc_feature 1..26: note = PCR_primers_fwd_seq
  source 1..26: mol_type = other DNA
ccaggtaacaaaccaaccaactttcg

SEQ ID NO: 26 - DNA, 24 bp, synthetic construct
  misc_feature 1..24: note = PCR_primers_rev_seq
  source 1..24: mol_type = other DNA
ggttactgccagttgaatctgagg

SEQ ID NO: 27 - DNA, 23 bp, synthetic construct
  misc_feature 1..23: note = PCR_primers_fwd_seq
  source 1..23: mol_type = other DNA
agcctcttctcgttcctcatcac

SEQ ID NO: 28 - DNA, 19 bp, synthetic construct
  misc_feature 1..19: note = PCR_primers_rev_seq
  source 1..19: mol_type = other DNA
ccgccattgccagccattc

SEQ ID NO: 29 - DNA, 21 bp, synthetic construct
  misc_feature 1..21: note = PCR_primers_fwd_seq
  source 1..21: mol_type = other DNA
ggagcgagatccctccaaaat

SEQ ID NO: 30 - DNA, 23 bp, synthetic construct
  misc_feature 1..23: note = PCR_primers_rev_seq
  source 1..23: mol_type = other DNA
ggctgttgtcatacttctcatgg

SEQ ID NO: 31 - RNA, 19 nt, synthetic construct
  misc_feature 1..19: note = target sequence in siRNA
  source 1..19: mol_type = other RNA
gtttgtttttcttgtttta

SEQ ID NO: 32 - RNA, 19 nt, synthetic construct
  misc_feature 1..19: note = target sequence in siRNA
  source 1..19: mol_type = other RNA
ccactagtctctagtcagt

SEQ ID NO: 33 - RNA, 19 nt, synthetic construct
  misc_feature 1..19: note = target sequence in siRNA
  source 1..19: mol_type = other RNA
ctctagtcagtgtgttaat

SEQ ID NO: 34 - RNA, 19 nt, synthetic construct
  misc_feature 1..19: note = target sequence in siRNA
  source 1..19: mol_type = other RNA
ctagtcagtgtgttaatct

SEQ ID NO: 35 - DNA, 21 bp, synthetic construct
  misc_feature 1..19: note = RNA
  source 1..21: mol_type = other DNA
  modified_base 2..4: mod_base = OTHER; note = uracil
  modified_base 6..10: mod_base = OTHER; note = uracil
  modified_base 12..13: mod_base = OTHER; note = uracil
  modified_base 15..18: mod_base = OTHER; note = uracil
  misc_feature 20..21: note = DNA
gtttgtttttcttgttttatt

SEQ ID NO: 36 - DNA, 21 bp, synthetic construct
  misc_feature 1..19: note = RNA
  source 1..21: mol_type = other DNA
  modified_base 1: mod_base = OTHER; note = uracil
  misc_feature 20..21: note = DNA
taaaacaagaaaaacaaactt

SEQ ID NO: 37 - DNA, 21 bp, synthetic construct
  misc_feature 1..19: note = RNA
  source 1..21: mol_type = other DNA
  modified_base 5: mod_base = OTHER; note = uracil
  modified_base 8: mod_base = OTHER; note = uracil
  modified_base 10: mod_base = OTHER; note = uracil
  modified_base 12: mod_base = OTHER; note = uracil
  modified_base 15: mod_base = OTHER; note = uracil
  modified_base 19: mod_base = OTHER; note = uracil
  misc_feature 20..21: note = DNA
ccactagtctctagtcagttt

SEQ ID NO: 38 - DNA, 21 bp, synthetic construct
  misc_feature 1..19: note = RNA
  source 1..21: mol_type = other DNA
  modified_base 3: mod_base = OTHER; note = uracil
  modified_base 7: mod_base = OTHER; note = uracil
  modified_base 14: mod_base = OTHER; note = uracil
  modified_base 17: mod_base = OTHER; note = uracil
  misc_feature 20..21: note = DNA
actgactagagactagtggtt

SEQ ID NO: 39 - DNA, 21 bp, synthetic construct
  misc_feature 1..19: note = RNA
  source 1..21: mol_type = other DNA
  modified_base 2: mod_base = OTHER; note = uracil
  modified_base 4: mod_base = OTHER; note = uracil
  modified_base 7: mod_base = OTHER; note = uracil
  modified_base 11: mod_base = OTHER; note = uracil
  modified_base 13: mod_base = OTHER; note = uracil
  modified_base 15..16: mod_base = OTHER; note = uracil
  modified_base 19: mod_base = OTHER; note = uracil
  misc_feature 20..21: note = DNA
ctctagtcagtgtgttaattt

SEQ ID NO: 40 - DNA, 21 bp, synthetic construct
  misc_feature 1..19: note = RNA
  source 1..21: mol_type = other DNA
  modified_base 2..3: mod_base = OTHER; note = uracil
  modified_base 11: mod_base = OTHER; note = uracil
  modified_base 15: mod_base = OTHER; note = uracil
  misc_feature 20..21: note = DNA
attaacacactgactagagtt

SEQ ID NO: 41 - DNA, 21 bp, synthetic construct
  misc_feature 1..19: note = RNA
  source 1..21: mol_type = other DNA
  modified_base 2: mod_base = OTHER; note = uracil
  modified_base 5: mod_base = OTHER; note = uracil
  modified_base 9: mod_base = OTHER; note = uracil
  modified_base 11: mod_base = OTHER; note = uracil
  modified_base 13..14: mod_base = OTHER; note = uracil
  modified_base 17: mod_base = OTHER; note = uracil
  modified_base 19: mod_base = OTHER; note = uracil
  misc_feature 20..21: note = DNA
ctagtcagtgtgttaatcttt

SEQ ID NO: 42 - DNA, 21 bp, synthetic construct
  misc_feature 1..19: note = RNA
  source 1..21: mol_type = other DNA
  modified_base 4..5: mod_base = OTHER; note = uracil
  modified_base 13: mod_base = OTHER; note = uracil
  modified_base 17: mod_base = OTHER; note = uracil
  misc_feature 20..21: note = DNA
agattaacacactgactagtt